European Patent Specification EP 3 737 664 B1, published April 10, 2024. Title: Compounds with Antimicrobial Activity. Applicant: The Hong Kong Polytechnic University The Chinese University of Hong Kong. Application EP 19739015.6. The sequence listing filed with the application follows.

SEQUENCE LISTING (28 sequences)

SEQ ID NO: 1 - DNA, 26 bp, Artificial Sequence
  Primer for B. subtilis nusB
aaaggagatctagacatgaaagaaga

SEQ ID NO: 2 - DNA, 23 bp, Artificial Sequence
  Primer for B. subtilis nusB
ttttctggtaccctatgattccc

SEQ ID NO: 3 - DNA, 29 bp, Artificial Sequence
  Primer for nusB mutants
ctttgcaggcactagctcaaattgatgtc

SEQ ID NO: 4 - DNA, 29 bp, Artificial Sequence
  Primer for nusB mutants
gacatcaatttgagctagtgcctgcaaag

SEQ ID NO: 5 - DNA, 29 bp, Artificial Sequence
  Primer for nusB mutants
gaattggaagctcgatgcgattgccaatg

SEQ ID NO: 6 - DNA, 29 bp, Artificial Sequence
  Primer for nusB mutants
cattggcaatcgcatcgagcttccaattc

SEQ ID NO: 7 - DNA, 29 bp, Artificial Sequence
  Primer for nusB mutants
gattgccaatgttgcccgtgcgattttgc

SEQ ID NO: 8 - DNA, 29 bp, Artificial Sequence
  Primer for nusB mutants
gcaaaatcgcacgggcaacattggcaatc

SEQ ID NO: 9 - DNA, 24 bp, Artificial Sequence
  Primer for B. subtilis nusE
aaggagggtctagaatggcaaaac

SEQ ID NO: 10 - DNA, 27 bp, Artificial Sequence
  Primer for B. subtilis nusE
ctatattttaggtaccaagtttaattt

SEQ ID NO: 11 - protein, 54 aa, Aquifex aeolicus
  misc_feature (25)..(27): Xaa is an unknown amino acid
  misc_feature (37)..(37): Xaa is an unknown amino acid
IDRLGYVERNALRLGVAELIFLKSXXXKEPGRVFIDXIVDLVKKYADEKAGKFV

SEQ ID NO: 12 - protein, 54 aa, Bacillus subtilis
  misc_feature (24)..(27): Xaa is an unknown amino acid
LDRIANVDRAILRLAAYEMAYAEXXXXDIPVNVSMNEAIELAKRFGDDKATKFV

SEQ ID NO: 13 - protein, 54 aa, Escherichia coli
  misc_feature (24)..(27): Xaa is an unknown amino acid
LEELGQVEKAVLRIALYELSKRSXXXXDVPYKVAINEAIELAKSFGAEDSHKFV

SEQ ID NO: 14 - protein, 54 aa, Haemophilus influenzae
  misc_feature (24)..(27): Xaa is an unknown amino acid
FDELDPIETAILRLAVYELRFELXXXXDVPYKVVINEAIEVAKVFGADESHKYI

SEQ ID NO: 15 - protein, 54 aa, Helicobacter pylori
  misc_feature (24)..(28): Xaa is an unknown amino acid
FKRLGSMEKAILRLGAYEIGFTPXXXXXTQNPIIINECIELGKLYAEPNTPKFL

SEQ ID NO: 16 - protein, 54 aa, Pseudomonas aeruginosa
  misc_feature (24)..(27): Xaa is an unknown amino acid
LAEIDPVELAILRLSTYELRNRIXXXXDVPYKVVINEGIELAKTFGATDGHKFV

SEQ ID NO: 17 - protein, 54 aa, Mycobacterium tuberculosis
  misc_feature (24)..(27): Xaa is an unknown amino acid
LDRLPAVDRAILRVSVWELLHAAXXXXDVPEPVVVDEAVQLAKELSTDDSPGFV

SEQ ID NO: 18 - protein, 54 aa, Staphylococcus aureus
  misc_feature (23)..(27): Xaa is an unknown amino acid
IARLLKTDRIILRMATYEILHSXXXXXDTPAKVVMNEAVELTKQFSDDDHYKFI

SEQ ID NO: 19 - protein, 54 aa, Streptococcus pneumoniae
  misc_feature (23)..(27): Xaa is an unknown amino acid
IERLTLVERNLLRLGVFEITSFXXXXXDTPQLVAVNEAIELAKDFSDQKSARFI

SEQ ID NO: 20 - protein, 48 aa, Aquifex aeolicus
GMEQEKIRIKLRAYDHRLLDQSVKQIIETVKRTGGVVKGPIPLPTRKS

SEQ ID NO: 21 - protein, 54 aa, Bacillus subtilis
MAKQKIRIRLKAYDHRILDQSAEKIVETAKRSGASVSGPIPLPTEKSVYTILRA

SEQ ID NO: 22 - protein, 54 aa, Escherichia coli
MQNQRIRIRLKAFDHRLIDQATAEIVETAKRTGAQVRGPIPLPTRKERFTVLIS

SEQ ID NO: 23 - protein, 54 aa, Haemophilus influenzae
MQNQRIRIRLKAFDHRLIDQSTAEIVETAKRTGAQVRGPIPLPTRKERFTVLIS

SEQ ID NO: 24 - protein, 52 aa, Helicobacter pylori
MEKIRLKLKAYDHRVLDRSVVAIVEAVKRSGSEIRGPIPLPTKNKRYTVLRS

SEQ ID NO: 25 - protein, 54 aa, Pseudomonas aeruginosa
MQNQQIRIRLKAFDHRLIDQSTQEIVETAKRTGAQVRGPIPLPTRKERFTVLIS

SEQ ID NO: 26 - protein, 54 aa, Mycobacterium tuberculosis
MAGQKIRIRLKAYDHEAIDASARKIVETVVRTGASVVGPVPLPTEKNVYCVIRS

SEQ ID NO: 27 - protein, 54 aa, Staphylococcus aureus
MAKQKIRIRLKAYDHRVIDQSAEKIVETAKRSGADVSGPIPLPTEKSVYTIIRA

SEQ ID NO: 28 - protein, 54 aa, Streptococcus pneumoniae
MANKKIRIRLKAYEHRTLDTAAAKIVESATRTGAQVAGPIPLPTERSLYTIIRA